European Patent Specification EP 3 755 811 B1, published April 2, 2025. Title: METHODS AND KITS FOR DETERMINING THE EFFICIENCY OF PLASMA SEPARATION FROM WHOLE BLOOD. Applicant: NUCLEIX LTD. The sequence listing filed with the application follows.

SEQUENCE LISTING (10 sequences)

SEQ ID NO: 1 - DNA, 126 bp, Homo sapiens
gtctttgtgacattgagttacagggctttgactcctgggtctaaaaattacaccaaatattgttaaatcttaaacactaacagcaattcaagcctcatcttcaggtcctggagaagatgccaatat

SEQ ID NO: 2 - DNA, 450 bp, Homo sapiens
gtcagcctttattatcactttgcaatacaaagaaagcaaggtgaagactaacttttctcttgtacagaatcatcaggctaaatttttggcattatttcagtccttggagacatctgagagattccgggatgccagtggtgcctctctggccacactgacaacaaataattcacctaaggaatagttcacttcagctattttttgctactcattggttgtcagtgccattgaggagagctcagtgtagatcaaagaaaacggtgtagatcaaagaaaacggtgattcggtgattgttccccttcttcccagccacccaccatctgaacctaatgcatcattgtacaatggccgtaaaggatgacaagggactcagcaatcagttcctggaggaaatgatgctgtggcttttggctggtggcaccatcatcctcagtcatcagtcagagtca

SEQ ID NO: 3 - DNA, 23 bp, Artificial Sequence
  Primer
gtctttgtgacattgagttacag

SEQ ID NO: 4 - DNA, 22 bp, Artificial Sequence
  Primer
atattggcatcttctccaggac

SEQ ID NO: 5 - DNA, 23 bp, Artificial Sequence
  Primer
gtcagcctttattatcactttgc

SEQ ID NO: 6 - DNA, 22 bp, Artificial Sequence
  Primer
tgactctgactgatgactgagg

SEQ ID NO: 7 - DNA, 520 bp, Homo sapiens
gatgcaatagtcagactgggaaaaggtagatgaatggaaaaggcaaacaggtctttatgaaaaacaatgcagatgatctctggtgtcacataatgtttattattattcagctatgtacatacttgaaaagatccattgtcattaaattattttttatgtcagcctttattatcactttgcaatacaaagaaagcaaggtgaagactaacttttctcttgtacagaatcatcaggctaaatttttggcattatttcagtccttggagacatctgagagattccgggatgccagtggtgcctctctggccacactgacaacaaataattcacctaaggaatagttcacttcagctattttttgctactcattggttgtcagtgccattgaggagagctcagtgtagatcaaagaaaacggtgtagatcaaagaaaacggtgattcggtgattgttccccttcttcccagccacccaccatctgaacctaatgcatcattgtacaatggccgtaaaggatgac

SEQ ID NO: 8 - DNA, 642 bp, Homo sapiens
atgaatggaaaaggcaaacaggtctttatgaaaaacaatgcagatgatctctggtgtcacataatgtttattattattcagctatgtacatacttgaaaagatccattgtcattaaattattttttatgtcagcctttattatcactttgcaatacaaagaaagcaaggtgaagactaacttttctcttgtacagaatcatcaggctaaatttttggcattatttcagtccttggagacatctgagagattccgggatgccagtggtgcctctctggccacactgacaacaaataattcacctaaggaatagttcacttcagctattttttgctactcattggttgtcagtgccattgaggagagctcagtgtagatcaaagaaaacggtgtagatcaaagaaaacggtgattcggtgattgttccccttcttcccagccacccaccatctgaacctaatgcatcattgtacaatggccgtaaaggatgacaagggactcagcaatcagttcctggaggaaatgatgctgtggcttttggctggtggcaccatcatcctcagtcatcagtcagagtcatcaaagtgatcattcatccattcactccctcctctgtctccaccccacagctaatcaactaacc

SEQ ID NO: 9 - DNA, 538 bp, Homo sapiens
tgaggtagagaaaagaatactcatgttaaagatagacatggaagatataaaaaagaccaaaatcaaacttctagagatgaaaaatgtataggatgggatcaatagcaaattagtgcaaaaaaagcaaacttgaaggcacagcaaaagaaaccatccaaaattaaaacaaagaaaaggttggaaaaacatataaagcatcaatgagttgaggaacaacttcaagcagtctaatatacatgtaaatttgagtcccagaaggaagaagtaagagtagactatagaaaatttattttaaggaatagcaaaaatttttccaaactgtatgtgaaaatagaaaactacatataaaaaatatgattacaaacccacagatccagtaagttcaacaaaccccaagcacagaacacatgaagaaagctaaaccaatgtaccctataattgaattgcacaaattcaatggtaaaaagaaaaatcttaaaagtagccagagtttttaaaaaaaaaaagaaagaaaaaagacacttaacatacagaggag

SEQ ID NO: 10 - DNA, 77 bp, Homo sapiens
agcaaggtgaagactaacttttctcttgtacagaatcatcaggctaaatttttggcattatttcagtccttggagac